European Patent Specification EP 3 747 909 B1, published March 4, 2026. Title: Anticancer drug. Applicant: OSAKA UNIVERSITY TOKYO INSTITUTE OF TECHNOLOGY. The sequence listing filed with the application follows.

SEQUENCE LISTING (2 sequences)

SEQ ID NO: 1 - DNA, 58 bp, Artificial Sequence
  shRNA1 targeting CD13 / APN
ccggccctcttcattcacttcagaactcgagttctgaagtgaatgaagagggtttttg

SEQ ID NO: 2 - DNA, 58 bp, Artificial Sequence
  shRNA2 targeting CD13 / APN
ccgggtgaccatagagtggtggaatctcgagattccaccactctatggtcactttttg